European Patent Application EP 4 691 562 A2, published February 11, 2026. Title: ANTI-PD-L1 COMBINATIONS FOR TREATING TUMORS. Applicant: Birdie Biopharmaceuticals Inc. Application EP 25209124.4, filed July 8, 2015. The sequence listing filed with the application follows.

SEQUENCE LISTING (10 sequences)

SEQ ID NO: 1 - DNA, 23 bp, synthetic construct
  source 1..23: mol_type = other DNA
cattgctgacaggatgcagaagg

SEQ ID NO: 2 - DNA, 22 bp, synthetic construct
  source 1..22: mol_type = other DNA
tgctggaaggtggacagtgagg

SEQ ID NO: 3 - DNA, 20 bp, synthetic construct
  source 1..20: mol_type = other DNA
ctccagcactgggtggaatg

SEQ ID NO: 4 - DNA, 20 bp, synthetic construct
  source 1..20: mol_type = other DNA
agtggagagcagttgaggac

SEQ ID NO: 5 - DNA, 20 bp, synthetic construct
  source 1..20: mol_type = other DNA
gtggcagagggagaatgtcg

SEQ ID NO: 6 - DNA, 23 bp, synthetic construct
  source 1..23: mol_type = other DNA
taaaacagcataaccttttgcga

SEQ ID NO: 7 - DNA, 23 bp, synthetic construct
  source 1..23: mol_type = other DNA
cctgagagagaagaaacacagcc

SEQ ID NO: 8 - DNA, 22 bp, synthetic construct
  source 1..22: mol_type = other DNA
ggctctccagacttctgctctg

SEQ ID NO: 9 - DNA, 21 bp, synthetic construct
  source 1..21: mol_type = other DNA
cagcaatggcctgggacctaa

SEQ ID NO: 10 - DNA, 20 bp, synthetic construct
  source 1..20: mol_type = other DNA
ggaaagccggcacaccaatc